European Patent Specification EP 3 519 061 B1, published March 29, 2023. Title: TOPICAL SLIMMING COSMETIC TREATMENT. Applicant: SEDERMA. The sequence listing filed with the application follows.

SEQUENCE LISTING (24 sequences)

SEQ ID NO: 1 - protein, 4 aa, artificial sequence
  synthetic peptide
RSRK

SEQ ID NO: 2 - protein, 4 aa, artificial sequence
  synthetic peptide
GQPR

SEQ ID NO: 3 - protein, 4 aa, artificial sequence
  synthetic peptide
KTFK

SEQ ID NO: 4 - protein, 4 aa, Artificial sequence
  Synthetic peptide
KTAK

SEQ ID NO: 5 - protein, 4 aa, Artificial sequence
  Synthetic peptide
KAYK

SEQ ID NO: 6 - protein, 4 aa, Artificial sequence
  Synthetic peptide
KFYK

SEQ ID NO: 7 - protein, 5 aa, artificial sequence
  synthetic peptide
KTTKS

SEQ ID NO: 8 - protein, 6 aa, artificial sequence
  Synthetic peptide
GKTTKS

SEQ ID NO: 9 - protein, 6 aa, artificial sequence
  synthetic peptide
VGVAPG

SEQ ID NO: 10 - protein, 4 aa, artificial sequence
  synthetic peptide
  MOD_RES (1)..(1): amidation by a Palmitoyl chain on the N terminal end
GQPR

SEQ ID NO: 11 - protein, 4 aa, Artificial sequence
  synthetic peptide
  MOD_RES (1)..(1): amidation by a Palmitoyl or Elaidoyl chain on the N terminal end
KTFK

SEQ ID NO: 12 - protein, 4 aa, Artificial sequence
  Synthetic peptide
  MOD_RES (1)..(1): amidation by a Elaidoyl chain on the N terminal end
KTAK

SEQ ID NO: 13 - protein, 4 aa, Artificial sequence
  Synthetic peptide
  MOD_RES (1)..(1): amidation by a Elaidoyl chain on the N terminal end
KAYK

SEQ ID NO: 14 - protein, 4 aa, Artificial sequence
  Synthetic peptide
  MOD_RES (1)..(1): amidation by a Elaidoyl chain on the N terminal end
KFYK

SEQ ID NO: 15 - protein, 5 aa, artificial sequence
  synthetic peptide
  MOD_RES (1)..(1): amidation by a Palmitoyl chain on the N terminal end
KTTKS

SEQ ID NO: 16 - protein, 5 aa, artificial sequence
  synthetic peptide
  MOD_RES (1)..(1): amidation by a Palmitoyl chain on the N terminal end
  MISC_FEATURE (5)..(5): Xaa being either a Proline P or a Leucine L.
YGGFX

SEQ ID NO: 17 - protein, 6 aa, Artificial sequence
  Synthetic peptide
  MOD_RES (1)..(1): amidation by a Palmitoyl chain on the N terminal end
  MISC_FEATURE (6)..(6): Xaa being Trp, Phe, Tyr, Tic, 7-hydroxy-Tic or Tpi
HLDIIX

SEQ ID NO: 18 - protein, 6 aa, artificial sequence
  synthetic peptide
  MOD_RES (1)..(1): amidation by a Palmitoyl chain on the N terminal end
VGVAPG

SEQ ID NO: 19 - protein, 6 aa, artificial sequence
  synthetic peptide
  MOD_RES (1)..(1): amidation by a Palmitoyl chain on the N terminal end
GKTTKS

SEQ ID NO: 20 - protein, 6 aa, artificial sequence
  synthetic peptide
  MOD_RES (1)..(1): Acetylation on the N-terminal end
EEMQRR

SEQ ID NO: 21 - protein, 5 aa, artificial sequence
  synthetic peptide
YAGFL

SEQ ID NO: 22 - protein, 4 aa, artificial sequence
  synthetic peptide
AHSH

SEQ ID NO: 23 - protein, 6 aa, artificial sequence
  synthetic peptide
SIKVAV

SEQ ID NO: 24 - protein, 6 aa, artificial sequence
  synthetic peptide
GPQGPQ